European Patent Application EP 4 342 908 A1, published March 27, 2024. Title: Chimeric Immunoglobulin. Applicant: Fapon Biotech Inc. Application CN202110674660.8. The sequence listing filed with the application follows.

SEQUENCE LISTING (8 sequences)

SEQ ID NO: 1 - DNA, 38 bp, Artificial Sequence
  Synthesized
gagagtcagtccttcccaaatgtcttccccctcgtctc

SEQ ID NO: 2 - DNA, 48 bp, Artificial Sequence
  Synthesized
cccgaattcttatcaatagcaggtgccacctgtgtcagacatgatcag

SEQ ID NO: 3 - protein, 455 aa, Artificial Sequence
  Synthesized
ESQSFPNVFPLVSCESPLSDKNLVAMGCLARDFLPSTISFTWNYQNNTEVIQGIRTFPTLRTGGKYLATSQVLLSPKSILEGSDEYLVCKIHYGGKNRDLHVPIPAVAEMNPNVNVFVPPRDGFSGPAPRKSKLICEATNFTPKPITVSWLKDGKLVESGFTTDPVTIENKGSTPQTYKVISTLTISEIDWLNLNVYTCRVDHRGLTFLKNVSSTCAASPSTDILTFTIPPSFADIFLSKSANLTCLVSNLATYETLNISWASQSGEPLETKIKIMESHPNGTFSAKGVASVCVEDWNNRKEFVCTVTHRDLPSPQKKFISKPNEVHKHPPAVYLLPPAREQLNLRESATVTCLVKGFSPADISVQWLQRGQLLPQEKYVTSAPMPEPGAPGFYFTHSILTVTEEEWNSGETYTCVVGHEALPHLVTERTVDKSTGKPTLYNVSLIMSDTGGTCY

SEQ ID NO: 4 - DNA, 39 bp, Artificial Sequence
  Synthesized
gagtctgcgagaaatcccaccatctacccactgacactc

SEQ ID NO: 5 - DNA, 42 bp, Artificial Sequence
  Synthesized
cccgaattctcagtagcagatgccatctccctctgacatgat

SEQ ID NO: 6 - protein, 344 aa, Artificial Sequence
  Synthesized
ESARNPTLYPLTLPPALSSDPVIIGCLIHDYFPSGTMNVTWGKSGKDITTVNFPPALASGGRYTMSSQLTLPAVECPEGESVKCSVQHDSNPVQELDVNCSGPTPPPPITIPSCQPSLSLQRPALEDLLLGSDASITCTLNGLRNPEGAVFTWEPSTGKDAVQKKAVQNSCGCYSVSSVLPGCAERWNSGASFKCTVTHPESGTLTGTIAKVTVNTFPPQVHLLPPPSEELALNELLSLTCLVRAFNPKEVLVRWLHGNEELSPESYLVFEPLKEPGEGATTYLVTSVLRVSAETWKQGDQYSCMVGHEALPMNFTQKTIDRLSGKPTNVSVSVIMSEGDGICY

SEQ ID NO: 7 - protein, 120 aa, Artificial Sequence
  Synthesized
QVQLQQPGAELVRPGASVKLSCKASGYSFTNYWMNWVKQRPGQGLEWIGMIHPSDSETRLNQKFKDKATLTVDKSSSTAYMQLSSLTAEDSAVYYCARSGDFYTYYFDYWGQGTTLTVSS

SEQ ID NO: 8 - protein, 225 aa, Artificial Sequence
  Synthesized
QVQLQQPGAELVRPGASVKLSCKASGYSFTNYWMNWVKQRPGQGLEWIGMIHPSDSETRLNQKFKDKATLTVDKSSSTAYMQLSSLTAEDSAVYYCARSGDFYTYYFDYWGQGTTLTVSSAKTTPPSVYPLAPGCGDTTGSSVTLGCLVKGYFPESVTVTWNSGSLSSSVHTFPALLQSGLYTMSSSVTVPSSTWPSQTVTCSVAHPASSTTVDKKLEPSGPIST